European Patent Application EP 4 545 646 A1, published April 30, 2025. Title: Verfahren zur Herstellung von D-Talitol. Applicant: Annikki GmbH. The sequence listing filed with the application follows.

SEQUENCE LISTING (4 sequences)

SEQ ID NO: 1 - DNA, 807 bp, synthetic construct
  source 1..807: mol_type = other DNA; note = oxidoreductase
atgaacgatcccgttctggaagccagaccgattttggagagatttcgcctcgacggccgcgtggcgctggtgaccggcggtgggcagggcatcggccgcgccttcgcccatgcgctgtgcgaggcaggcgccgcagtggccgtcgtcgatctgcgcctggacctggccgaggaagtggcgcatgagctggtaaacaagcagatcgacgccatcgcaattcaggccgatgtgacgaagcccgatcaggtgcagacgatggttgatgccattctgtccaggtgggggacgttgacgatcggtgtcaacaacgccggcatcggcttgtgggcggatgccgaaagcatggcatacacagactggctgcgcgtgatcgatattgatctgaactcggttttcctctgcgcccaggctgaagcgagggtcatgctgccggccggctacggcaagatcatcaacacggcgtcgatgtccggccatatcagcaacacgccgcaaaatcaggctgcttacaacacggccaaggctggcgtgatccatctgacgcgcagccttgccgcggaatgggccaagcggggagtgcgcgtcaacagcatcagccccggctatacgcgcaccaaattggttgacgacctgctcgccacgccgatcggacagacgatgttgcccacctggatgggcatgacgcccatgggacgaatggccgaggtcaccgatctgcaaggcgccgtcgtctacctggcgtcgtcggcgtccgactatatgaccggccatgacatggtgattgacggcggctattgttgctggtaa

SEQ ID NO: 2 - protein, 268 aa, synthetic construct
  source 1..268: note = oxidoreductase
MNDPVLEARPILERFRLDGRVALVTGGGQGIGRAFAHALCEAGAAVAVVDLRLDLAEEVAHELVNKQIDAIAIQADVTKPDQVQTMVDAILSRWGTLTIGVNNAGIGLWADAESMAYTDWLRVIDIDLNSVFLCAQAEARVMLPAGYGKIINTASMSGHISNTPQNQAAYNTAKAGVIHLTRSLAAEWAKRGVRVNSISPGYTRTKLVDDLLATPIGQTMLPTWMGMTPMGRMAEVTDLQGAVVYLASSASDYMTGHDMVIDGGYCCW

SEQ ID NO: 3 - DNA, 1206 bp, synthetic construct
  source 1..1206: mol_type = other DNA; note = formate dehydrogenase
atggcgaaaatactttgcgttctctatgacgatccggtcgacggctacccgaagacctatgcgcgcgacgacctgccgaagatcgaccactatccgggcgggcagacgctgcccacgcccaaggcgatcgacttcacgccgggcgcgctgctcggctcggtctccggcgagctcggcctgcgcaaatacctggaagccaacggccataccttcgtcgtcacctccgataaggacggcccggattcggtgttcgagagggaactcgtcgacgccgacgtggtgatctcgcagcccttctggccggcctatctgacgcccgagcgcatcgccaaggcgaagaacctgaagctcgcgctcaccgccggcatcggctccgatcatgtcgatcttcagtcagctatcgaccgtggcatcactgtggccgaagtcacatattgcaactcgatcagcgtcgccgagcacgtggtgatgatgatcctcggcctggtacgaaactacattccctcgcatgactgggcgcgcaagggcggctggaacatagccgactgcgtagagcactcctacgacctcgagggcatgaccgtcggctcggtggccgccggccgcatcggcctcgccgtgctgcgccgcctcgcgccgttcgacgtgaagctgcactataccgaccgccaccgtctgccagaagcggtcgagaaggagctgggcctcgtctggcacgatacccgcgaggacatgtacccgcattgcgacgtggtcacgctcaacgtgccgctgcaccccgaaaccgagcacatgatcaatgacgagacgctgaagctgttcaagcgcggcgcctatatcgtcaacaccgcccgcggcaagctcgccgaccgcgacgccatcgtccgcgcgatcgagagcgggcagctcgcgggctatgccggcgacgtgtggttcccgcagccggctccgaaggaccacccctggcgcaccatgaagtgggaaggcatgacgccgcacatctccggcacctcgctctctgcccaggcgcgctacgcggcgggcacgcgcgagatcctcgaatgcttcttcgagggccggccgatccgcgacgagtacctgatcgtgcagggcggcgcgctcgccggcaccggcgcgcattcctactcgaagggcaatgcgaccggcggttcggaagaggccgcgaagttcaagaaggctggctga

SEQ ID NO: 4 - protein, 401 aa, synthetic construct
  source 1..401: note = formate dehydrogenase
MAKILCVLYDDPVDGYPKTYARDDLPKIDHYPGGQTLPTPKAIDFTPGALLGSVSGELGLRKYLEANGHTFVVTSDKDGPDSVFERELVDADVVISQPFWPAYLTPERIAKAKNLKLALTAGIGSDHVDLQSAIDRGITVAEVTYCNSISVAEHVVMMILGLVRNYIPSHDWARKGGWNIADCVEHSYDLEGMTVGSVAAGRIGLAVLRRLAPFDVKLHYTDRHRLPEAVEKELGLVWHDTREDMYPHCDVVTLNVPLHPETEHMINDETLKLFKRGAYIVNTARGKLADRDAIVRAIESGQLAGYAGDVWFPQPAPKDHPWRTMKWEGMTPHISGTSLSAQARYAAGTREILECFFEGRPIRDEYLIVQGGALAGTGAHSYSKGNATGGSEEAAKFKKAG